European Patent Specification EP 4 392 176 B1, published February 18, 2026. Title: CONTROLLED CELL-CELL INTERACTION ASSAY. Applicant: Singleron Biotechnologies Inc. The sequence listing filed with the application follows.

SEQUENCE LISTING (101 sequences)

SEQ ID NO: 1 - DNA, 40 bp, synthetic construct
  misc_feature 1..40: note = Synthetic Oligonucleotide
  misc_difference 1: note = 5' Phosphorylation
  misc_feature 40: note = n is a, c, g, or t
  source 1..40: mol_type = other DNA
aggccagagcattcgaacgtgattttttttttttttttvn

SEQ ID NO: 2 - DNA, 40 bp, synthetic construct
  misc_feature 1..40: note = Synthetic Oligonucleotide
  misc_difference 1: note = 5' Phosphorylation
  misc_feature 40: note = n is a, c, g, or t
  source 1..40: mol_type = other DNA
aggccagagcattcgaaacatcgtttttttttttttttvn

SEQ ID NO: 3 - DNA, 40 bp, synthetic construct
  misc_feature 1..40: note = Synthetic Oligonucleotide
  misc_difference 1: note = 5' Phosphorylation
  misc_feature 40: note = n is a, c, g, or t
  source 1..40: mol_type = other DNA
aggccagagcattcgatgcctaatttttttttttttttvn

SEQ ID NO: 4 - DNA, 40 bp, synthetic construct
  misc_feature 1..40: note = Synthetic Oligonucleotide
  misc_difference 1: note = 5' Phosphorylation
  misc_feature 40: note = n is a, c, g, or t
  source 1..40: mol_type = other DNA
aggccagagcattcgagtggtcatttttttttttttttvn

SEQ ID NO: 5 - DNA, 40 bp, synthetic construct
  misc_feature 1..40: note = Synthetic Oligonucleotide
  misc_difference 1: note = 5' Phosphorylation
  misc_feature 40: note = n is a, c, g, or t
  source 1..40: mol_type = other DNA
aggccagagcattcgaccactgttttttttttttttttvn

SEQ ID NO: 6 - DNA, 40 bp, synthetic construct
  misc_feature 1..40: note = Synthetic Oligonucleotide
  misc_difference 1: note = 5' Phosphorylation
  misc_feature 40: note = n is a, c, g, or t
  source 1..40: mol_type = other DNA
aggccagagcattcgacattggctttttttttttttttvn

SEQ ID NO: 7 - DNA, 40 bp, synthetic construct
  misc_feature 1..40: note = Synthetic Oligonucleotide
  misc_difference 1: note = 5' Phosphorylation
  misc_feature 40: note = n is a, c, g, or t
  source 1..40: mol_type = other DNA
aggccagagcattcgcagatctgtttttttttttttttvn

SEQ ID NO: 8 - DNA, 40 bp, synthetic construct
  misc_feature 1..40: note = Synthetic Oligonucleotide
  misc_difference 1: note = 5' Phosphorylation
  misc_feature 40: note = n is a, c, g, or t
  source 1..40: mol_type = other DNA
aggccagagcattcgcatcaagttttttttttttttttvn

SEQ ID NO: 9 - DNA, 40 bp, synthetic construct
  misc_feature 1..40: note = Synthetic Oligonucleotide
  misc_difference 1: note = 5' Phosphorylation
  misc_feature 40: note = n is a, c, g, or t
  source 1..40: mol_type = other DNA
aggccagagcattcgcgctgatctttttttttttttttvn

SEQ ID NO: 10 - DNA, 40 bp, synthetic construct
  misc_feature 1..40: note = Synthetic Oligonucleotide
  misc_difference 1: note = 5' Phosphorylation
  misc_feature 40: note = n is a, c, g, or t
  source 1..40: mol_type = other DNA
aggccagagcattcgacaagctatttttttttttttttvn

SEQ ID NO: 11 - DNA, 40 bp, synthetic construct
  misc_feature 1..40: note = Synthetic Oligonucleotide
  misc_difference 1: note = 5' Phosphorylation
  misc_feature 40: note = n is a, c, g, or t
  source 1..40: mol_type = other DNA
aggccagagcattcgctgtagcctttttttttttttttvn

SEQ ID NO: 12 - DNA, 40 bp, synthetic construct
  misc_feature 1..40: note = Synthetic Oligonucleotide
  misc_difference 1: note = 5' Phosphorylation
  misc_feature 40: note = n is a, c, g, or t
  source 1..40: mol_type = other DNA
aggccagagcattcgagtacaagtttttttttttttttvn

SEQ ID NO: 13 - DNA, 40 bp, synthetic construct
  misc_feature 1..40: note = Synthetic Oligonucleotide
  misc_difference 1: note = 5' Phosphorylation
  misc_feature 40: note = n is a, c, g, or t
  source 1..40: mol_type = other DNA
aggccagagcattcgaacaaccatttttttttttttttvn

SEQ ID NO: 14 - DNA, 40 bp, synthetic construct
  misc_feature 1..40: note = Synthetic Oligonucleotide
  misc_difference 1: note = 5' Phosphorylation
  misc_feature 40: note = n is a, c, g, or t
  source 1..40: mol_type = other DNA
aggccagagcattcgaaccgagatttttttttttttttvn

SEQ ID NO: 15 - DNA, 40 bp, synthetic construct
  misc_feature 1..40: note = Synthetic Oligonucleotide
  misc_difference 1: note = 5' Phosphorylation
  misc_feature 40: note = n is a, c, g, or t
  source 1..40: mol_type = other DNA
aggccagagcattcgaacgcttatttttttttttttttvn

SEQ ID NO: 16 - DNA, 40 bp, synthetic construct
  misc_feature 1..40: note = Synthetic Oligonucleotide
  misc_difference 1: note = 5' Phosphorylation
  misc_feature 40: note = n is a, c, g, or t
  source 1..40: mol_type = other DNA
aggccagagcattcgaagacggatttttttttttttttvn

SEQ ID NO: 17 - DNA, 40 bp, synthetic construct
  misc_feature 1..40: note = Synthetic Oligonucleotide
  misc_difference 1: note = 5' Phosphorylation
  misc_feature 40: note = n is a, c, g, or t
  source 1..40: mol_type = other DNA
aggccagagcattcgaaggtacatttttttttttttttvn

SEQ ID NO: 18 - DNA, 40 bp, synthetic construct
  misc_feature 1..40: note = Synthetic Oligonucleotide
  misc_difference 1: note = 5' Phosphorylation
  misc_feature 40: note = n is a, c, g, or t
  source 1..40: mol_type = other DNA
aggccagagcattcgacacagaatttttttttttttttvn

SEQ ID NO: 19 - DNA, 40 bp, synthetic construct
  misc_feature 1..40: note = Synthetic Oligonucleotide
  misc_difference 1: note = 5' Phosphorylation
  misc_feature 40: note = n is a, c, g, or t
  source 1..40: mol_type = other DNA
aggccagagcattcgacagcagatttttttttttttttvn

SEQ ID NO: 20 - DNA, 40 bp, synthetic construct
  misc_feature 1..40: note = Synthetic Oligonucleotide
  misc_difference 1: note = 5' Phosphorylation
  misc_feature 40: note = n is a, c, g, or t
  source 1..40: mol_type = other DNA
aggccagagcattcgacctccaatttttttttttttttvn

SEQ ID NO: 21 - DNA, 40 bp, synthetic construct
  misc_feature 1..40: note = Synthetic Oligonucleotide
  misc_difference 1: note = 5' Phosphorylation
  misc_feature 40: note = n is a, c, g, or t
  source 1..40: mol_type = other DNA
aggccagagcattcgacgctcgatttttttttttttttvn

SEQ ID NO: 22 - DNA, 40 bp, synthetic construct
  misc_feature 1..40: note = Synthetic Oligonucleotide
  misc_difference 1: note = 5' Phosphorylation
  misc_feature 40: note = n is a, c, g, or t
  source 1..40: mol_type = other DNA
aggccagagcattcgacgtatcatttttttttttttttvn

SEQ ID NO: 23 - DNA, 40 bp, synthetic construct
  misc_feature 1..40: note = Synthetic Oligonucleotide
  misc_difference 1: note = 5' Phosphorylation
  misc_feature 40: note = n is a, c, g, or t
  source 1..40: mol_type = other DNA
aggccagagcattcgactatgcatttttttttttttttvn

SEQ ID NO: 24 - DNA, 40 bp, synthetic construct
  misc_feature 1..40: note = Synthetic Oligonucleotide
  misc_difference 1: note = 5' Phosphorylation
  misc_feature 40: note = n is a, c, g, or t
  source 1..40: mol_type = other DNA
aggccagagcattcgagagtcaatttttttttttttttvn

SEQ ID NO: 25 - DNA, 40 bp, synthetic construct
  misc_feature 1..40: note = Synthetic Oligonucleotide
  misc_difference 1: note = 5' Phosphorylation
  misc_feature 40: note = n is a, c, g, or t
  source 1..40: mol_type = other DNA
aggccagagcattcgagatcgcatttttttttttttttvn

SEQ ID NO: 26 - DNA, 40 bp, synthetic construct
  misc_feature 1..40: note = Synthetic Oligonucleotide
  misc_difference 1: note = 5' Phosphorylation
  misc_feature 40: note = n is a, c, g, or t
  source 1..40: mol_type = other DNA
aggccagagcattcgagcaggaatttttttttttttttvn

SEQ ID NO: 27 - DNA, 40 bp, synthetic construct
  misc_feature 1..40: note = Synthetic Oligonucleotide
  misc_difference 1: note = 5' Phosphorylation
  misc_feature 40: note = n is a, c, g, or t
  source 1..40: mol_type = other DNA
aggccagagcattcgagtcactatttttttttttttttvn

SEQ ID NO: 28 - DNA, 40 bp, synthetic construct
  misc_feature 1..40: note = Synthetic Oligonucleotide
  misc_difference 1: note = 5' Phosphorylation
  misc_feature 40: note = n is a, c, g, or t
  source 1..40: mol_type = other DNA
aggccagagcattcgatcctgtatttttttttttttttvn

SEQ ID NO: 29 - DNA, 40 bp, synthetic construct
  misc_feature 1..40: note = Synthetic Oligonucleotide
  misc_difference 1: note = 5' Phosphorylation
  misc_feature 40: note = n is a, c, g, or t
  source 1..40: mol_type = other DNA
aggccagagcattcgattgaggatttttttttttttttvn

SEQ ID NO: 30 - DNA, 40 bp, synthetic construct
  misc_feature 1..40: note = Synthetic Oligonucleotide
  misc_difference 1: note = 5' Phosphorylation
  misc_feature 40: note = n is a, c, g, or t
  source 1..40: mol_type = other DNA
aggccagagcattcgcaaccacatttttttttttttttvn

SEQ ID NO: 31 - DNA, 40 bp, synthetic construct
  misc_feature 1..40: note = Synthetic Oligonucleotide
  misc_difference 1: note = 5' Phosphorylation
  misc_feature 40: note = n is a, c, g, or t
  source 1..40: mol_type = other DNA
aggccagagcattcggactagtatttttttttttttttvn

SEQ ID NO: 32 - DNA, 40 bp, synthetic construct
  misc_feature 1..40: note = Synthetic Oligonucleotide
  misc_difference 1: note = 5' Phosphorylation
  misc_feature 40: note = n is a, c, g, or t
  source 1..40: mol_type = other DNA
aggccagagcattcgcaatggaatttttttttttttttvn

SEQ ID NO: 33 - DNA, 40 bp, synthetic construct
  misc_feature 1..40: note = Synthetic Oligonucleotide
  misc_difference 1: note = 5' Phosphorylation
  misc_feature 40: note = n is a, c, g, or t
  source 1..40: mol_type = other DNA
aggccagagcattcgcacttcgatttttttttttttttvn

SEQ ID NO: 34 - DNA, 40 bp, synthetic construct
  misc_feature 1..40: note = Synthetic Oligonucleotide
  misc_difference 1: note = 5' Phosphorylation
  misc_feature 40: note = n is a, c, g, or t
  source 1..40: mol_type = other DNA
aggccagagcattcgcagcgttatttttttttttttttvn

SEQ ID NO: 35 - DNA, 40 bp, synthetic construct
  misc_feature 1..40: note = Synthetic Oligonucleotide
  misc_difference 1: note = 5' Phosphorylation
  misc_feature 40: note = n is a, c, g, or t
  source 1..40: mol_type = other DNA
aggccagagcattcgcataccaatttttttttttttttvn

SEQ ID NO: 36 - DNA, 40 bp, synthetic construct
  misc_feature 1..40: note = Synthetic Oligonucleotide
  misc_difference 1: note = 5' Phosphorylation
  misc_feature 40: note = n is a, c, g, or t
  source 1..40: mol_type = other DNA
aggccagagcattcgccagttcatttttttttttttttvn

SEQ ID NO: 37 - DNA, 40 bp, synthetic construct
  misc_feature 1..40: note = Synthetic Oligonucleotide
  misc_difference 1: note = 5' Phosphorylation
  misc_feature 40: note = n is a, c, g, or t
  source 1..40: mol_type = other DNA
aggccagagcattcgccgaagtatttttttttttttttvn

SEQ ID NO: 38 - DNA, 40 bp, synthetic construct
  misc_feature 1..40: note = Synthetic Oligonucleotide
  misc_difference 1: note = 5' Phosphorylation
  misc_feature 40: note = n is a, c, g, or t
  source 1..40: mol_type = other DNA
aggccagagcattcgccgtgagatttttttttttttttvn

SEQ ID NO: 39 - DNA, 40 bp, synthetic construct
  misc_feature 1..40: note = Synthetic Oligonucleotide
  misc_difference 1: note = 5' Phosphorylation
  misc_feature 40: note = n is a, c, g, or t
  source 1..40: mol_type = other DNA
aggccagagcattcgcctcctgatttttttttttttttvn

SEQ ID NO: 40 - DNA, 40 bp, synthetic construct
  misc_feature 1..40: note = Synthetic Oligonucleotide
  misc_difference 1: note = 5' Phosphorylation
  misc_feature 40: note = n is a, c, g, or t
  source 1..40: mol_type = other DNA
aggccagagcattcgcgaacttatttttttttttttttvn

SEQ ID NO: 41 - DNA, 40 bp, synthetic construct
  misc_feature 1..40: note = Synthetic Oligonucleotide
  misc_difference 1: note = 5' Phosphorylation
  misc_feature 40: note = n is a, c, g, or t
  source 1..40: mol_type = other DNA
aggccagagcattcgcgactggatttttttttttttttvn

SEQ ID NO: 42 - DNA, 40 bp, synthetic construct
  misc_feature 1..40: note = Synthetic Oligonucleotide
  misc_difference 1: note = 5' Phosphorylation
  misc_feature 40: note = n is a, c, g, or t
  source 1..40: mol_type = other DNA
aggccagagcattcgcgcatacatttttttttttttttvn

SEQ ID NO: 43 - DNA, 40 bp, synthetic construct
  misc_feature 1..40: note = Synthetic Oligonucleotide
  misc_difference 1: note = 5' Phosphorylation
  misc_feature 40: note = n is a, c, g, or t
  source 1..40: mol_type = other DNA
aggccagagcattcgctcaatgatttttttttttttttvn

SEQ ID NO: 44 - DNA, 40 bp, synthetic construct
  misc_feature 1..40: note = Synthetic Oligonucleotide
  misc_difference 1: note = 5' Phosphorylation
  misc_feature 40: note = n is a, c, g, or t
  source 1..40: mol_type = other DNA
aggccagagcattcgctgagccatttttttttttttttvn

SEQ ID NO: 45 - DNA, 40 bp, synthetic construct
  misc_feature 1..40: note = Synthetic Oligonucleotide
  misc_difference 1: note = 5' Phosphorylation
  misc_feature 40: note = n is a, c, g, or t
  source 1..40: mol_type = other DNA
aggccagagcattcgctggcatatttttttttttttttvn

SEQ ID NO: 46 - DNA, 40 bp, synthetic construct
  misc_feature 1..40: note = Synthetic Oligonucleotide
  misc_difference 1: note = 5' Phosphorylation
  misc_feature 40: note = n is a, c, g, or t
  source 1..40: mol_type = other DNA
aggccagagcattcggaatctgatttttttttttttttvn

SEQ ID NO: 47 - DNA, 40 bp, synthetic construct
  misc_feature 1..40: note = Synthetic Oligonucleotide
  misc_difference 1: note = 5' Phosphorylation
  misc_feature 40: note = n is a, c, g, or t
  source 1..40: mol_type = other DNA
aggccagagcattcgcaagactatttttttttttttttvn

SEQ ID NO: 48 - DNA, 40 bp, synthetic construct
  misc_feature 1..40: note = Synthetic Oligonucleotide
  misc_difference 1: note = 5' Phosphorylation
  misc_feature 40: note = n is a, c, g, or t
  source 1..40: mol_type = other DNA
aggccagagcattcggagctgaatttttttttttttttvn

SEQ ID NO: 49 - DNA, 40 bp, synthetic construct
  misc_feature 1..40: note = Synthetic Oligonucleotide
  misc_difference 1: note = 5' Phosphorylation
  misc_feature 40: note = n is a, c, g, or t
  source 1..40: mol_type = other DNA
aggccagagcattcggatagacatttttttttttttttvn

SEQ ID NO: 50 - DNA, 40 bp, synthetic construct
  misc_feature 1..40: note = Synthetic Oligonucleotide
  misc_difference 1: note = 5' Phosphorylation
  misc_feature 40: note = n is a, c, g, or t
  source 1..40: mol_type = other DNA
aggccagagcattcggccacatatttttttttttttttvn

SEQ ID NO: 51 - DNA, 55 bp, synthetic construct
  misc_feature 1..55: note = Synthetic Oligonucleotide
  misc_difference 1: note = 5' Biotin
  misc_feature 23..32: note = n is a, c, g, or t
  source 1..55: mol_type = other DNA
caagcgttggcttctcgcatctnnnnnnnnnnaacgtgatatccacgtgcttgag

SEQ ID NO: 52 - DNA, 55 bp, synthetic construct
  misc_feature 1..55: note = Synthetic Oligonucleotide
  misc_difference 1: note = 5' Biotin
  misc_feature 23..32: note = n is a, c, g, or t
  source 1..55: mol_type = other DNA
caagcgttggcttctcgcatctnnnnnnnnnnaaacatcgatccacgtgcttgag

SEQ ID NO: 53 - DNA, 55 bp, synthetic construct
  misc_feature 1..55: note = Synthetic Oligonucleotide
  misc_difference 1: note = 5' Biotin
  misc_feature 23..32: note = n is a, c, g, or t
  source 1..55: mol_type = other DNA
caagcgttggcttctcgcatctnnnnnnnnnnatgcctaaatccacgtgcttgag

SEQ ID NO: 54 - DNA, 55 bp, synthetic construct
  misc_feature 1..55: note = Synthetic Oligonucleotide
  misc_difference 1: note = 5' Biotin
  misc_feature 23..32: note = n is a, c, g, or t
  source 1..55: mol_type = other DNA
caagcgttggcttctcgcatctnnnnnnnnnnagtggtcaatccacgtgcttgag

SEQ ID NO: 55 - DNA, 55 bp, synthetic construct
  misc_feature 1..55: note = Synthetic Oligonucleotide
  misc_difference 1: note = 5' Biotin
  misc_feature 23..32: note = n is a, c, g, or t
  source 1..55: mol_type = other DNA
caagcgttggcttctcgcatctnnnnnnnnnnaccactgtatccacgtgcttgag

SEQ ID NO: 56 - DNA, 55 bp, synthetic construct
  misc_feature 1..55: note = Synthetic Oligonucleotide
  misc_difference 1: note = 5' Biotin
  misc_feature 23..32: note = n is a, c, g, or t
  source 1..55: mol_type = other DNA
caagcgttggcttctcgcatctnnnnnnnnnnacattggcatccacgtgcttgag

SEQ ID NO: 57 - DNA, 55 bp, synthetic construct
  misc_feature 1..55: note = Synthetic Oligonucleotide
  misc_difference 1: note = 5' Biotin
  misc_feature 23..32: note = n is a, c, g, or t
  source 1..55: mol_type = other DNA
caagcgttggcttctcgcatctnnnnnnnnnncagatctgatccacgtgcttgag

SEQ ID NO: 58 - DNA, 55 bp, synthetic construct
  misc_feature 1..55: note = Synthetic Oligonucleotide
  misc_difference 1: note = 5' Biotin
  misc_feature 23..32: note = n is a, c, g, or t
  source 1..55: mol_type = other DNA
caagcgttggcttctcgcatctnnnnnnnnnncatcaagtatccacgtgcttgag

SEQ ID NO: 59 - DNA, 55 bp, synthetic construct
  misc_feature 1..55: note = Synthetic Oligonucleotide
  misc_difference 1: note = 5' Biotin
  misc_feature 23..32: note = n is a, c, g, or t
  source 1..55: mol_type = other DNA
caagcgttggcttctcgcatctnnnnnnnnnncgctgatcatccacgtgcttgag

SEQ ID NO: 60 - DNA, 55 bp, synthetic construct
  misc_feature 1..55: note = Synthetic Oligonucleotide
  misc_difference 1: note = 5' Biotin
  misc_feature 23..32: note = n is a, c, g, or t
  source 1..55: mol_type = other DNA
caagcgttggcttctcgcatctnnnnnnnnnnacaagctaatccacgtgcttgag

SEQ ID NO: 61 - DNA, 55 bp, synthetic construct
  misc_feature 1..55: note = Synthetic Oligonucleotide
  misc_difference 1: note = 5' Biotin
  misc_feature 23..32: note = n is a, c, g, or t
  source 1..55: mol_type = other DNA
caagcgttggcttctcgcatctnnnnnnnnnnctgtagccatccacgtgcttgag

SEQ ID NO: 62 - DNA, 55 bp, synthetic construct
  misc_feature 1..55: note = Synthetic Oligonucleotide
  misc_difference 1: note = 5' Biotin
  misc_feature 23..32: note = n is a, c, g, or t
  source 1..55: mol_type = other DNA
caagcgttggcttctcgcatctnnnnnnnnnnagtacaagatccacgtgcttgag

SEQ ID NO: 63 - DNA, 55 bp, synthetic construct
  misc_feature 1..55: note = Synthetic Oligonucleotide
  misc_difference 1: note = 5' Biotin
  misc_feature 23..32: note = n is a, c, g, or t
  source 1..55: mol_type = other DNA
caagcgttggcttctcgcatctnnnnnnnnnnaacaaccaatccacgtgcttgag

SEQ ID NO: 64 - DNA, 55 bp, synthetic construct
  misc_feature 1..55: note = Synthetic Oligonucleotide
  misc_difference 1: note = 5' Biotin
  misc_feature 23..32: note = n is a, c, g, or t
  source 1..55: mol_type = other DNA
caagcgttggcttctcgcatctnnnnnnnnnnaaccgagaatccacgtgcttgag

SEQ ID NO: 65 - DNA, 55 bp, synthetic construct
  misc_feature 1..55: note = Synthetic Oligonucleotide
  misc_difference 1: note = 5' Biotin
  misc_feature 23..32: note = n is a, c, g, or t
  source 1..55: mol_type = other DNA
caagcgttggcttctcgcatctnnnnnnnnnnaacgcttaatccacgtgcttgag

SEQ ID NO: 66 - DNA, 55 bp, synthetic construct
  misc_feature 1..55: note = Synthetic Oligonucleotide
  misc_difference 1: note = 5' Biotin
  misc_feature 23..32: note = n is a, c, g, or t
  source 1..55: mol_type = other DNA
caagcgttggcttctcgcatctnnnnnnnnnnaagacggaatccacgtgcttgag

SEQ ID NO: 67 - DNA, 55 bp, synthetic construct
  misc_feature 1..55: note = Synthetic Oligonucleotide
  misc_difference 1: note = 5' Biotin
  misc_feature 23..32: note = n is a, c, g, or t
  source 1..55: mol_type = other DNA
caagcgttggcttctcgcatctnnnnnnnnnnaaggtacaatccacgtgcttgag

SEQ ID NO: 68 - DNA, 55 bp, synthetic construct
  misc_feature 1..55: note = Synthetic Oligonucleotide
  misc_difference 1: note = 5' Biotin
  misc_feature 23..32: note = n is a, c, g, or t
  source 1..55: mol_type = other DNA
caagcgttggcttctcgcatctnnnnnnnnnnacacagaaatccacgtgcttgag

SEQ ID NO: 69 - DNA, 55 bp, synthetic construct
  misc_feature 1..55: note = Synthetic Oligonucleotide
  misc_difference 1: note = 5' Biotin
  misc_feature 23..32: note = n is a, c, g, or t
  source 1..55: mol_type = other DNA
caagcgttggcttctcgcatctnnnnnnnnnnacagcagaatccacgtgcttgag

SEQ ID NO: 70 - DNA, 55 bp, synthetic construct
  misc_feature 1..55: note = Synthetic Oligonucleotide
  misc_difference 1: note = 5' Biotin
  misc_feature 23..32: note = n is a, c, g, or t
  source 1..55: mol_type = other DNA
caagcgttggcttctcgcatctnnnnnnnnnnacctccaaatccacgtgcttgag

SEQ ID NO: 71 - DNA, 55 bp, synthetic construct
  misc_feature 1..55: note = Synthetic Oligonucleotide
  misc_difference 1: note = 5' Biotin
  misc_feature 23..32: note = n is a, c, g, or t
  source 1..55: mol_type = other DNA
caagcgttggcttctcgcatctnnnnnnnnnnacgctcgaatccacgtgcttgag

SEQ ID NO: 72 - DNA, 55 bp, synthetic construct
  misc_feature 1..55: note = Synthetic Oligonucleotide
  misc_difference 1: note = 5' Biotin
  misc_feature 23..32: note = n is a, c, g, or t
  source 1..55: mol_type = other DNA
caagcgttggcttctcgcatctnnnnnnnnnnacgtatcaatccacgtgcttgag

SEQ ID NO: 73 - DNA, 55 bp, synthetic construct
  misc_feature 1..55: note = Synthetic Oligonucleotide
  misc_difference 1: note = 5' Biotin
  misc_feature 23..32: note = n is a, c, g, or t
  source 1..55: mol_type = other DNA
caagcgttggcttctcgcatctnnnnnnnnnnactatgcaatccacgtgcttgag

SEQ ID NO: 74 - DNA, 55 bp, synthetic construct
  misc_feature 1..55: note = Synthetic Oligonucleotide
  misc_difference 1: note = 5' Biotin
  misc_feature 23..32: note = n is a, c, g, or t
  source 1..55: mol_type = other DNA
caagcgttggcttctcgcatctnnnnnnnnnnagagtcaaatccacgtgcttgag

SEQ ID NO: 75 - DNA, 55 bp, synthetic construct
  misc_feature 1..55: note = Synthetic Oligonucleotide
  misc_difference 1: note = 5' Biotin
  misc_feature 23..32: note = n is a, c, g, or t
  source 1..55: mol_type = other DNA
caagcgttggcttctcgcatctnnnnnnnnnnagatcgcaatccacgtgcttgag

SEQ ID NO: 76 - DNA, 55 bp, synthetic construct
  misc_feature 1..55: note = Synthetic Oligonucleotide
  misc_difference 1: note = 5' Biotin
  misc_feature 23..32: note = n is a, c, g, or t
  source 1..55: mol_type = other DNA
caagcgttggcttctcgcatctnnnnnnnnnnagcaggaaatccacgtgcttgag

SEQ ID NO: 77 - DNA, 55 bp, synthetic construct
  misc_feature 1..55: note = Synthetic Oligonucleotide
  misc_difference 1: note = 5' Biotin
  misc_feature 23..32: note = n is a, c, g, or t
  source 1..55: mol_type = other DNA
caagcgttggcttctcgcatctnnnnnnnnnnagtcactaatccacgtgcttgag

SEQ ID NO: 78 - DNA, 55 bp, synthetic construct
  misc_feature 1..55: note = Synthetic Oligonucleotide
  misc_difference 1: note = 5' Biotin
  misc_feature 23..32: note = n is a, c, g, or t
  source 1..55: mol_type = other DNA
caagcgttggcttctcgcatctnnnnnnnnnnatcctgtaatccacgtgcttgag

SEQ ID NO: 79 - DNA, 55 bp, synthetic construct
  misc_feature 1..55: note = Synthetic Oligonucleotide
  misc_difference 1: note = 5' Biotin
  misc_feature 23..32: note = n is a, c, g, or t
  source 1..55: mol_type = other DNA
caagcgttggcttctcgcatctnnnnnnnnnnattgaggaatccacgtgcttgag

SEQ ID NO: 80 - DNA, 55 bp, synthetic construct
  misc_feature 1..55: note = Synthetic Oligonucleotide
  misc_difference 1: note = 5' Biotin
  misc_feature 23..32: note = n is a, c, g, or t
  source 1..55: mol_type = other DNA
caagcgttggcttctcgcatctnnnnnnnnnncaaccacaatccacgtgcttgag

SEQ ID NO: 81 - DNA, 55 bp, synthetic construct
  misc_feature 1..55: note = Synthetic Oligonucleotide
  misc_difference 1: note = 5' Biotin
  misc_feature 23..32: note = n is a, c, g, or t
  source 1..55: mol_type = other DNA
caagcgttggcttctcgcatctnnnnnnnnnngactagtaatccacgtgcttgag

SEQ ID NO: 82 - DNA, 55 bp, synthetic construct
  misc_feature 1..55: note = Synthetic Oligonucleotide
  misc_difference 1: note = 5' Biotin
  misc_feature 23..32: note = n is a, c, g, or t
  source 1..55: mol_type = other DNA
caagcgttggcttctcgcatctnnnnnnnnnncaatggaaatccacgtgcttgag

SEQ ID NO: 83 - DNA, 55 bp, synthetic construct
  misc_feature 1..55: note = Synthetic Oligonucleotide
  misc_difference 1: note = 5' Biotin
  misc_feature 23..32: note = n is a, c, g, or t
  source 1..55: mol_type = other DNA
caagcgttggcttctcgcatctnnnnnnnnnncacttcgaatccacgtgcttgag

SEQ ID NO: 84 - DNA, 55 bp, synthetic construct
  misc_feature 1..55: note = Synthetic Oligonucleotide
  misc_difference 1: note = 5' Biotin
  misc_feature 23..32: note = n is a, c, g, or t
  source 1..55: mol_type = other DNA
caagcgttggcttctcgcatctnnnnnnnnnncagcgttaatccacgtgcttgag

SEQ ID NO: 85 - DNA, 55 bp, synthetic construct
  misc_feature 1..55: note = Synthetic Oligonucleotide
  misc_difference 1: note = 5' Biotin
  misc_feature 23..32: note = n is a, c, g, or t
  source 1..55: mol_type = other DNA
caagcgttggcttctcgcatctnnnnnnnnnncataccaaatccacgtgcttgag

SEQ ID NO: 86 - DNA, 55 bp, synthetic construct
  misc_feature 1..55: note = Synthetic Oligonucleotide
  misc_difference 1: note = 5' Biotin
  misc_feature 23..32: note = n is a, c, g, or t
  source 1..55: mol_type = other DNA
caagcgttggcttctcgcatctnnnnnnnnnnccagttcaatccacgtgcttgag

SEQ ID NO: 87 - DNA, 55 bp, synthetic construct
  misc_feature 1..55: note = Synthetic Oligonucleotide
  misc_difference 1: note = 5' Biotin
  misc_feature 23..32: note = n is a, c, g, or t
  source 1..55: mol_type = other DNA
caagcgttggcttctcgcatctnnnnnnnnnnccgaagtaatccacgtgcttgag

SEQ ID NO: 88 - DNA, 55 bp, synthetic construct
  misc_feature 1..55: note = Synthetic Oligonucleotide
  misc_difference 1: note = 5' Biotin
  misc_feature 23..32: note = n is a, c, g, or t
  source 1..55: mol_type = other DNA
caagcgttggcttctcgcatctnnnnnnnnnnccgtgagaatccacgtgcttgag

SEQ ID NO: 89 - DNA, 55 bp, synthetic construct
  misc_feature 1..55: note = Synthetic Oligonucleotide
  misc_difference 1: note = 5' Biotin
  misc_feature 23..32: note = n is a, c, g, or t
  source 1..55: mol_type = other DNA
caagcgttggcttctcgcatctnnnnnnnnnncctcctgaatccacgtgcttgag

SEQ ID NO: 90 - DNA, 55 bp, synthetic construct
  misc_feature 1..55: note = Synthetic Oligonucleotide
  misc_difference 1: note = 5' Biotin
  misc_feature 23..32: note = n is a, c, g, or t
  source 1..55: mol_type = other DNA
caagcgttggcttctcgcatctnnnnnnnnnncgaacttaatccacgtgcttgag

SEQ ID NO: 91 - DNA, 55 bp, synthetic construct
  misc_feature 1..55: note = Synthetic Oligonucleotide
  misc_difference 1: note = 5' Biotin
  misc_feature 23..32: note = n is a, c, g, or t
  source 1..55: mol_type = other DNA
caagcgttggcttctcgcatctnnnnnnnnnncgactggaatccacgtgcttgag

SEQ ID NO: 92 - DNA, 55 bp, synthetic construct
  misc_feature 1..55: note = Synthetic Oligonucleotide
  misc_difference 1: note = 5' Biotin
  misc_feature 23..32: note = n is a, c, g, or t
  source 1..55: mol_type = other DNA
caagcgttggcttctcgcatctnnnnnnnnnncgcatacaatccacgtgcttgag

SEQ ID NO: 93 - DNA, 55 bp, synthetic construct
  misc_feature 1..55: note = Synthetic Oligonucleotide
  misc_difference 1: note = 5' Biotin
  misc_feature 23..32: note = n is a, c, g, or t
  source 1..55: mol_type = other DNA
caagcgttggcttctcgcatctnnnnnnnnnnctcaatgaatccacgtgcttgag

SEQ ID NO: 94 - DNA, 55 bp, synthetic construct
  misc_feature 1..55: note = Synthetic Oligonucleotide
  misc_difference 1: note = 5' Biotin
  misc_feature 23..32: note = n is a, c, g, or t
  source 1..55: mol_type = other DNA
caagcgttggcttctcgcatctnnnnnnnnnnctgagccaatccacgtgcttgag

SEQ ID NO: 95 - DNA, 55 bp, synthetic construct
  misc_feature 1..55: note = Synthetic Oligonucleotide
  misc_difference 1: note = 5' Biotin
  misc_feature 23..32: note = n is a, c, g, or t
  source 1..55: mol_type = other DNA
caagcgttggcttctcgcatctnnnnnnnnnnctggcataatccacgtgcttgag

SEQ ID NO: 96 - DNA, 55 bp, synthetic construct
  misc_feature 1..55: note = Synthetic Oligonucleotide
  misc_difference 1: note = 5' Biotin
  misc_feature 23..32: note = n is a, c, g, or t
  source 1..55: mol_type = other DNA
caagcgttggcttctcgcatctnnnnnnnnnngaatctgaatccacgtgcttgag

SEQ ID NO: 97 - DNA, 55 bp, synthetic construct
  misc_feature 1..55: note = Synthetic Oligonucleotide
  misc_difference 1: note = 5' Biotin
  misc_feature 23..32: note = n is a, c, g, or t
  source 1..55: mol_type = other DNA
caagcgttggcttctcgcatctnnnnnnnnnncaagactaatccacgtgcttgag

SEQ ID NO: 98 - DNA, 55 bp, synthetic construct
  misc_feature 1..55: note = Synthetic Oligonucleotide
  misc_difference 1: note = 5' Biotin
  misc_feature 23..32: note = n is a, c, g, or t
  source 1..55: mol_type = other DNA
caagcgttggcttctcgcatctnnnnnnnnnngagctgaaatccacgtgcttgag

SEQ ID NO: 99 - DNA, 55 bp, synthetic construct
  misc_feature 1..55: note = Synthetic Oligonucleotide
  misc_difference 1: note = 5' Biotin
  misc_feature 23..32: note = n is a, c, g, or t
  source 1..55: mol_type = other DNA
caagcgttggcttctcgcatctnnnnnnnnnngatagacaatccacgtgcttgag

SEQ ID NO: 100 - DNA, 55 bp, synthetic construct
  misc_feature 1..55: note = Synthetic Oligonucleotide
  misc_difference 1: note = 5' Biotin
  misc_feature 23..32: note = n is a, c, g, or t
  source 1..55: mol_type = other DNA
caagcgttggcttctcgcatctnnnnnnnnnngccacataatccacgtgcttgag

SEQ ID NO: 101 - DNA, 30 bp, synthetic construct
  misc_feature 1..30: note = Synthetic Oligonucleotide
  source 1..30: mol_type = other DNA
cgaatgctctggcctctcaagcacgtggat